European Patent Specification EP 3 664 832 B1, published October 18, 2023. Title: Truncated Guinea Pig L-Asparaginase Variants and Methods of Use. Applicant: The Board of Trustees of the University of Illinois Lavie, Arnon Nguyen, Hien-Anh Shalk, Amanda. The sequence listing filed with the application follows.

SEQUENCE LISTING (94 sequences)

SEQ ID NO: 1 - protein, 565 aa, Cavia porcellus
MARASGSERHLLLIYTGGTLGMQSKGGVLVPGPGLVTLLRTLPMFHDKEFAQAQGLPDHALALPPASHGPRVLYTVLECQPLLDSSDMTIDDWIRIAKIIERHYEQYQGFVVIHGTDTMASGASMLSFMLENLHKPVILTGAQVPIRVLWNDARENLLGALLVAGQYIIPEVCLFMNSQLFRGNRVTKVDSQKFEAFCSPNLSPLATVGADVTIAWDLVRKVKWKDPLVVHSNMEHDVALLRLYPGIPASLVRAFLQPPLKGVVLETFGSGNGPSKPDLLQELRAAAQRGLIMVNCSQCLRGSVTPGYATSLAGANIVSGLDMTSEAALAKLSYVLGLPELSLERRQELLAKDLRGEMTLPTADLHQSSPPGSTLGQGVARLFSLFGCQEEDSVQDAVMPSLALALAHAGELEALQALMELGSDLRLKDSNGQTLLHVAARNGRDGVVTMLLHRGMDVNARDRDGLSPLLLAVQGRHRECIRLLRKAGACLSPQDLKDAGTELCRLASRADMEGLQAWGQAGADLQQPGYDGRSALCVAEAAGNQEVLALLRNLALVGPEVPPAI

SEQ ID NO: 2 - protein, 573 aa, Homo sapiens
MARAVGPERRLLAVYTGGTIGMRSELGVLVPGTGLAAILRTLPMFHDEEHARARGLSEDTLVLPPASRNQRILYTVLECQPLFDSSDMTIAEWVCLAQTIKRHYEQYHGFVVIHGTDTMAFAASMLSFMLENLQKTVILTGAQVPIHALWSDGRENLLGALLMAGQYVIPEVCLFFQNQLFRGNRATKVDARRFAAFCSPNLLPLATVGADITINRELVRKVDGKAGLVVHSSMEQDVGLLRLYPGIPAALVRAFLQPPLKGVVMETFGSGNGPTKPDLLQELRVATERGLVIVNCTHCLQGAVTTDYAAGMAMAGAGVISGFDMTSEAALAKLSYVLGQPGLSLDVRKELLTKDLRGEMTPPSVEERRPSLQGNTLGGGVSWLLSLSGSQEADALRNALVPSLACAAAHAGDVEALQALVELGSDLGLVDFNGQTPLHAAARGGHTEAVTMLLQRGVDVNTRDTDGFSPLLLAVRGRHPGVIGLLREAGASLSTQELEEAGTELCRLAYRADLEGLQVWWQAGADLGQPGYDGHSALHVAEAAGNLAVVAFLQSLEGAVGAQAPCPEVLPGV

SEQ ID NO: 3 - protein, 359 aa, Artificial Sequence
  Synthetic polypeptide
MARASGSERHLLLIYTGGTLGMQSKGGVLVPGPGLVTLLRTLPMFHDKEFAQAQGLPDHALALPPASHGPRVLYTVLECQPLLDSSDMTIDDWIRIAKIIERHYEQYQGFVVIHGTDTMASGASMLSFMLENLHKPVILTGAQVPIRVLWNDARENLLGALLVAGQYIIPEVCLFMNSQLFRGNRVTKVDSQKFEAFCSPNLSPLATVGADVTIAWDLVRKVKWKDPLVVHSNMEHDVALLRLYPGIPASLVRAFLQPPLKGVVLETFGSGNGPSKPDLLQELRAAAQRGLIMVNCSQCLRGSVTPGYATSLAGANIVSGLDMTSEAALAKLSYVLGLPELSLERRQELLAKDLRGEMT

SEQ ID NO: 4 - protein, 367 aa, Artificial Sequence
  Synthetic polypeptide
MARASGSERHLLLIYTGGTLGMQSKGGVLVPGPGLVTLLRTLPMFHDKEFAQAQGLPDHALALPPASHGPRVLYTVLECQPLLDSSDMTIDDWIRIAKIIERHYEQYQGFVVIHGTDTMASGASMLSFMLENLHKPVILTGAQVPIRVLWNDARENLLGALLVAGQYIIPEVCLFMNSQLFRGNRVTKVDSQKFEAFCSPNLSPLATVGADVTIAWDLVRKVKWKDPLVVHSNMEHDVALLRLYPGIPASLVRAFLQPPLKGVVLETFGSGNGPSKPDLLQELRAAAQRGLIMVNCSQCLRGSVTPGYATSLAGANIVSGLDMTSEAALAKLSYVLGLPELSLERRQELLAKDLRGEMTLPTADLHQ

SEQ ID NO: 5 - protein, 369 aa, Artificial Sequence
  Synthetic polypeptide
MARASGSERHLLLIYTGGTLGMQSKGGVLVPGPGLVTLLRTLPMFHDKEFAQAQGLPDHALALPPASHGPRVLYTVLECQPLLDSSDMTIDDWIRIAKIIERHYEQYQGFVVIHGTDTMASGASMLSFMLENLHKPVILTGAQVPIRVLWNDARENLLGALLVAGQYIIPEVCLFMNSQLFRGNRVTKVDSQKFEAFCSPNLSPLATVGADVTIAWDLVRKVKWKDPLVVHSNMEHDVALLRLYPGIPASLVRAFLQPPLKGVVLETFGSGNGPSKPDLLQELRAAAQRGLIMVNCSQCLRGSVTPGYATSLAGANIVSGLDMTSEAALAKLSYVLGLPELSLERRQELLAKDLRGEMTLPTADLHQSS

SEQ ID NO: 6 - protein, 374 aa, Artificial Sequence
  Synthetic polypeptide
MARASGSERHLLLIYTGGTLGMQSKGGVLVPGPGLVTLLRTLPMFHDKEFAQAQGLPDHALALPPASHGPRVLYTVLECQPLLDSSDMTIDDWIRIAKIIERHYEQYQGFVVIHGTDTMASGASMLSFMLENLHKPVILTGAQVPIRVLWNDARENLLGALLVAGQYIIPEVCLFMNSQLFRGNRVTKVDSQKFEAFCSPNLSPLATVGADVTIAWDLVRKVKWKDPLVVHSNMEHDVALLRLYPGIPASLVRAFLQPPLKGVVLETFGSGNGPSKPDLLQELRAAAQRGLIMVNCSQCLRGSVTPGYATSLAGANIVSGLDMTSEAALAKLSYVLGLPELSLERRQELLAKDLRGEMTLPTADLHQSSPPGST

SEQ ID NO: 7 - protein, 384 aa, Artificial Sequence
  Synthetic polypeptide
MARASGSERHLLLIYTGGTLGMQSKGGVLVPGPGLVTLLRTLPMFHDKEFAQAQGLPDHALALPPASHGPRVLYTVLECQPLLDSSDMTIDDWIRIAKIIERHYEQYQGFVVIHGTDTMASGASMLSFMLENLHKPVILTGAQVPIRVLWNDARENLLGALLVAGQYIIPEVCLFMNSQLFRGNRVTKVDSQKFEAFCSPNLSPLATVGADVTIAWDLVRKVKWKDPLVVHSNMEHDVALLRLYPGIPASLVRAFLQPPLKGVVLETFGSGNGPSKPDLLQELRAAAQRGLIMVNCSQCLRGSVTPGYATSLAGANIVSGLDMTSEAALAKLSYVLGLPELSLERRQELLAKDLRGEMTLPTADLHQSSPPGSTLGQGVARLFS

SEQ ID NO: 8 - protein, 392 aa, Artificial Sequence
  Synthetic polypeptide
MARASGSERHLLLIYTGGTLGMQSKGGVLVPGPGLVTLLRTLPMFHDKEFAQAQGLPDHALALPPASHGPRVLYTVLECQPLLDSSDMTIDDWIRIAKIIERHYEQYQGFVVIHGTDTMASGASMLSFMLENLHKPVILTGAQVPIRVLWNDARENLLGALLVAGQYIIPEVCLFMNSQLFRGNRVTKVDSQKFEAFCSPNLSPLATVGADVTIAWDLVRKVKWKDPLVVHSNMEHDVALLRLYPGIPASLVRAFLQPPLKGVVLETFGSGNGPSKPDLLQELRAAAQRGLIMVNCSQCLRGSVTPGYATSLAGANIVSGLDMTSEAALAKLSYVLGLPELSLERRQELLAKDLRGEMTLPTADLHQSSPPGSTLGQGVARLFSLFGCQEED

SEQ ID NO: 9 - protein, 396 aa, Artificial Sequence
  Synthetic polypeptide
MARASGSERHLLLIYTGGTLGMQSKGGVLVPGPGLVTLLRTLPMFHDKEFAQAQGLPDHALALPPASHGPRVLYTVLECQPLLDSSDMTIDDWIRIAKIIERHYEQYQGFVVIHGTDTMASGASMLSFMLENLHKPVILTGAQVPIRVLWNDARENLLGALLVAGQYIIPEVCLFMNSQLFRGNRVTKVDSQKFEAFCSPNLSPLATVGADVTIAWDLVRKVKWKDPLVVHSNMEHDVALLRLYPGIPASLVRAFLQPPLKGVVLETFGSGNGPSKPDLLQELRAAAQRGLIMVNCSQCLRGSVTPGYATSLAGANIVSGLDMTSEAALAKLSYVLGLPELSLERRQELLAKDLRGEMTLPTADLHQSSPPGSTLGQGVARLFSLFGCQEEDSVQD

SEQ ID NO: 10 - DNA, 33 bp, Artificial Sequence
  Synthetic oligonucleotide
aacgtcggatccttaaatagccggcgggacttc

SEQ ID NO: 11 - DNA, 24 bp, Artificial Sequence
  Synthetic oligonucleotide
atggcacgcgcttcgggctcggaa

SEQ ID NO: 12 - DNA, 19 bp, Artificial Sequence
  Synthetic oligonucleotide
ccagattacgcagcagagc

SEQ ID NO: 13 - DNA, 21 bp, Artificial Sequence
  Synthetic oligonucleotide
gctcgtgctgtgggtccggaa

SEQ ID NO: 14 - DNA, 18 bp, Artificial Sequence
  Synthetic oligonucleotide
gacacccggcagcacttc

SEQ ID NO: 15 - DNA, 44 bp, Artificial Sequence
  Synthetic oligonucleotide
ctgatgcaggtctgccgtcggcagcgtcatttcaccgcgcaggt

SEQ ID NO: 16 - DNA, 43 bp, Artificial Sequence
  Synthetic oligonucleotide
aaggacctgcgcggtgaaatgacgctgccgacggcagacctgc

SEQ ID NO: 17 - DNA, 45 bp, Artificial Sequence
  Synthetic oligonucleotide
gcgacgttcttccacagacggcggggtcatttcaccacgcagatc

SEQ ID NO: 18 - DNA, 44 bp, Artificial Sequence
  Synthetic oligonucleotide
aaagatctgcgtggtgaaatgaccccgccgtctgtggaagaacg

SEQ ID NO: 19 - DNA, 48 bp, Artificial Sequence
  Synthetic oligonucleotide
  misc_feature (22)..(23): n is a, c, g, or t
  misc_feature (25)..(26): n is a, c, g, or t
tacaccggcggcaccattggcnnknnkagtgagctcggcgtgcttgtg

SEQ ID NO: 20 - DNA, 48 bp, Artificial Sequence
  Synthetic oligonucleotide
  misc_feature (23)..(24): n is a, c, g, or t
  misc_feature (26)..(27): n is a, c, g, or t
cacaagcacgccgagctcactmnnmnngccaatggtgccgccggtgta

SEQ ID NO: 21 - DNA, 51 bp, Artificial Sequence
  Synthetic oligonucleotide
  misc_feature (22)..(23): n is a, c, g, or t
  misc_feature (28)..(29): n is a, c, g, or t
ctggagtgccagcccctcttcnnktccnnkgacatgaccatcgctgagtgg

SEQ ID NO: 22 - DNA, 51 bp, Artificial Sequence
  Synthetic oligonucleotide
  misc_feature (23)..(24): n is a, c, g, or t
  misc_feature (29)..(30): n is a, c, g, or t
ccactcagcgatggtcatgtcmnnggamnngaagaggggctggcactccag

SEQ ID NO: 23 - DNA, 54 bp, Artificial Sequence
  Synthetic oligonucleotide
  misc_feature (25)..(26): n is a, c, g, or t
  misc_feature (28)..(29): n is a, c, g, or t
cagtaccacggctttgtggtcatcnnknnkaccgacaccatggcctttgctgcc

SEQ ID NO: 24 - DNA, 54 bp, Artificial Sequence
  Synthetic oligonucleotide
  misc_feature (26)..(27): n is a, c, g, or t
  misc_feature (29)..(30): n is a, c, g, or t
ggcagcaaaggccatggtgtcggtmnnmnngatgaccacaaagccgtggtactg

SEQ ID NO: 25 - DNA, 53 bp, Artificial Sequence
  Synthetic oligonucleotide
  misc_feature (24)..(25): n is a, c, g, or t
  misc_feature (27)..(28): n is a, c, g, or t
  misc_feature (30)..(31): n is a, c, g, or t
agaagactgtcatcctcactgggnnknnknnkcccatccatgccctgtggagc

SEQ ID NO: 26 - DNA, 52 bp, Artificial Sequence
  Synthetic oligonucleotide
  misc_feature (22)..(23): n is a, c, g, or t
  misc_feature (25)..(26): n is a, c, g, or t
  misc_feature (28)..(29): n is a, c, g, or t
gctccacagggcatgatgggmnnmnnmnncccagtgaggatgacagtcttct

SEQ ID NO: 27 - DNA, 52 bp, Artificial Sequence
  Synthetic oligonucleotide
  misc_feature (24)..(25): n is a, c, g, or t
  misc_feature (27)..(28): n is a, c, g, or t
gcaaccgggcaaccaaggtagacnnknnkaggttcgcagctttctgctcccc

SEQ ID NO: 28 - DNA, 52 bp, Artificial Sequence
  Synthetic oligonucleotide
  misc_feature (25)..(26): n is a, c, g, or t
  misc_feature (28)..(29): n is a, c, g, or t
ggggagcagaaagctgcgaacctmnnmnngtctaccttggttgcccggttgc

SEQ ID NO: 29 - DNA, 47 bp, Artificial Sequence
  Synthetic oligonucleotide
  misc_feature (18)..(19): n is a, c, g, or t
  misc_feature (27)..(28): n is a, c, g, or t
tcatccacggcaccgacnnkatggccnnkgctgcctcgatgctgtcc

SEQ ID NO: 30 - DNA, 47 bp, Artificial Sequence
  Synthetic oligonucleotide
  misc_feature (20)..(21): n is a, c, g, or t
  misc_feature (29)..(30): n is a, c, g, or t
ggacagcatcgaggcagcmnnggccatmnngtcggtgccgtggatga

SEQ ID NO: 31 - DNA, 63 bp, Artificial Sequence
  Synthetic oligonucleotide
  misc_feature (19)..(20): n is a, c, g, or t
  misc_feature (31)..(32): n is a, c, g, or t
  misc_feature (43)..(44): n is a, c, g, or t
tccagtgacatgaccatcnnkgagtgggttnnkcttgcccagnnkatcaagaggcactacgag

SEQ ID NO: 32 - DNA, 63 bp, Artificial Sequence
  Synthetic oligonucleotide
  misc_feature (20)..(21): n is a, c, g, or t
  misc_feature (32)..(33): n is a, c, g, or t
  misc_feature (44)..(45): n is a, c, g, or t
ctcgtagtgcctcttgatmnnctgggcaagmnnaacccactcmnngatggtcatgtcactgga

SEQ ID NO: 33 - DNA, 48 bp, Artificial Sequence
  Synthetic oligonucleotide
  misc_feature (19)..(20): n is a, c, g, or t
  misc_feature (25)..(26): n is a, c, g, or t
  misc_feature (28)..(29): n is a, c, g, or t
ggcggcaccattggcatgnnkagtnnknnkggcgtgcttgtgcccggg

SEQ ID NO: 34 - DNA, 48 bp, Artificial Sequence
  Synthetic oligonucleotide
  misc_feature (20)..(21): n is a, c, g, or t
  misc_feature (23)..(24): n is a, c, g, or t
  misc_feature (29)..(30): n is a, c, g, or t
cccgggcacaagcacgccmnnmnnactmnncatgccaatggtgccgcc

SEQ ID NO: 35 - DNA, 1722 bp, Artificial Sequence
  Synthetic polynucleotide
atggctcgtgctgtgggtccggaacgccgcctgctggctgtctatacgggtggtacgattggtatgcgctctgaactgggtgtcctggtgccgggtaccggtctggcagcaattctgcgtacgctgccgatgtttcatgatgaagaacacgcacgtgcacgcggtctgtcggaagacaccctggtgctgccgccggcaagccgtaaccagcgcatcctgtataccgttctggaatgccaaccgctgtttgatagctctgacatgaccattgccgaatgggtttgtctggcacagacgatcaaacgtcattatgaacaataccacggtttcgtggttattcatggcaccgatacgatggcctttgcagcttccatgctgtcattcatgctggaaaacctgcagaagaccgttattctgacgggcgctcaagtcccgatccacgcactgtggagcgacggtcgcgaaaatctgctgggcgccctgctgatggcaggccagtatgtcatcccggaagtgtgcctgtttttccagaaccaactgttccgtggtaatcgcgctaccaaagtcgatgcgcgtcgctttgcggccttctgtagcccgaacctgctgccgctggctaccgttggtgcagatattacgatcaatcgtgaactggtgcgcaaagttgacggcaaggcaggtctggtcgtgcatagttccatggaacaggatgtcggcctgctgcgtctgtacccgggtattccggcagctctggtgcgtgcctttctgcagccgccgctgaaaggtgttgtcatggaaaccttcggttctggcaacggtccgacgaagccggatctgctgcaggaactgcgtgtggcaaccgaacgcggcctggtcattgtgaattgcacgcactgtctgcaaggcgcagttaccacggattatgcagccggtatggcaatggctggtgcgggtgtcatctcgggttttgacatgaccagcgaagcagctctggcgaaactgtcctacgttctgggccagccgggtctgtcactggatgtccgtaaagaactgctgaccaaggacctgcgcggtgaaatgacgccgccgtctgtggaagaacgtcgcccgagtctgcagggtaacaccctgggcggtggcgtttcttggctgctgtcactgtcgggcagccaagaagccgatgcactgcgcaatgcactggtgccgagtctggcatgcgcagcagcacatgcaggtgacgtggaagctctgcaggcgctggttgaactgggttccgatctgggcctggtggactttaacggtcaaaccccgctgcatgctgcagcacgtggtggccacaccgaagcagttacgatgctgctgcagcgtggcgttgatgtcaatacccgcgatacggacggtttcagtccgctgctgctggcagtccgtggtcgtcatccgggcgtgatcggtctgctgcgcgaagctggtgcgtctctgagtacccaggaactggaagaagcgggcacggaactgtgtcgtctggcctatcgcgcagatctggaaggcctgcaagtgtggtggcaagcaggtgcagatctgggtcagccgggttacgacggtcatagcgccctgcacgttgcagaagcagctggtaatctggctgtggttgcgtttctgcaaagtctggaaggtgccgtcggtgcccaagcgccgtgcccggaagtgctgccgggtgtctaa

SEQ ID NO: 36 - DNA, 1698 bp, Artificial Sequence
  Synthetic polynucleotide
atggcacgcgcttcgggctcggaacgtcatctgctgctgatctacacgggtggcacgctgggtatgcaatccaagggtggtgttctggtcccgggtccgggtctggtgaccctgctgcgtacgctgccgatgtttcatgataaagaattcgcacaggcacaaggcctgccggaccatgctctggcgctgccgccggcctctcacggtccgcgcgtgctgtataccgttctggaatgccagccgctgctggatagctctgacatgacgattgatgactggattcgtatcgcgaagattatcgaacgccattatgaacagtaccaaggttttgtggttatccacggcaccgatacgatggcttcaggcgcgtcgatgctgagcttcatgctggaaaacctgcacaaaccggtgattctgaccggtgcccaggtcccgatccgtgtgctgtggaacgatgcacgcgaaaatctgctgggtgccctgctggttgcaggccagtatattatcccggaagtctgcctgtttatgaactcgcaactgttccgtggcaatcgcgtcacgaaggtggatagccagaaatttgaagcattctgttctccgaacctgagtccgctggctaccgttggtgcggatgtcacgattgcgtgggacctggttcgtaaagtcaagtggaaagatccgctggtcgtgcattccaatatggaacacgacgtcgcactgctgcgtctgtacccgggcatcccggctagcctggttcgtgcgtttctgcagccgccgctgaagggtgttgtcctggaaaccttcggctccggtaatggcccgtcaaaaccggatctgctgcaggaactgcgtgcagcagcacaacgcggcctgattatggtgaactgctcgcagtgtctgcgcggtagcgttaccccgggttatgccacgagcctggcaggtgcaaatatcgtgtctggcctggatatgaccagtgaagctgcgctggcgaagctgtcttacgttctgggcctgccggaactgagtctggaacgtcgccaggaactgctggctaaagatctgcgtggtgaaatgaccctgccgacggcagacctgcatcagagttccccgccgggctccaccctgggtcaaggcgtggcccgcctgttttcactgttcggttgtcaggaagaagattcggtgcaagacgcagttatgccgagcctggctctggcactggcacacgcaggtgaactggaagccctgcaagcactgatggaactgggttccgatctgcgtctgaaagactcaaacggccagaccctgctgcatgttgccgcacgtaatggtcgcgatggcgtggttacgatgctgctgcaccgcggtatggacgtgaacgcacgtgatcgtgacggtctgtcaccgctgctgctggcagttcaaggtcgtcatcgcgaatgcattcgtctgctgcgcaaggctggcgcgtgtctgtctccgcaggatctgaaagacgcgggtaccgaactgtgccgtctggctagtcgcgcggatatggaaggtctgcaggcatggggtcaagcaggtgcagatctgcagcaaccgggttacgacggccgtagtgccctgtgtgtggcagaagctgcgggtaatcaggaagtgctggctctgctgcgtaatctggctctggttggcccggaagtcccgccggctatttaa

SEQ ID NO: 37 - protein, 571 aa, Artificial Sequence
  Synthetic polypeptide
MARASGSERHLLLIYTGGTLGMQSKGGVLVPGPGLVTLLRTLPMFHDKEFAQAQGLPDHALALPPASHGPRVLYTVLECQPLLDSSDMTIDDWIRIAKIIERHYEQYQGFVVIHGTDTMASGASMLSFMLENLHKPVILTGAQVPIRVLWNDARENLLGALLVAGQYIIPEVCLFMNSQLFRGNRVTKVDSQKFEAFCSPNLSPLATVGADVTIAWDLVRKVKWKDPLVVHSSMEQDVGLLRLYPGIPASLVRAFLQPPLKGVVLETFGSGNGPSKPDLLQELRAAAERGLIMVNCSQCLRGSVTPGYATSLAGANIVSGLDMTSEAALAKLSYVLGLPELSLERRQELLAKDLRGEMTPPSVEERRPSLQGNTLGGGVSWLLSLSGSQEADALRNALVPSLACAAAHAGDVEALQALVELGSDLGLVDFNGQTPLHAAARGGHTEAVTMLLQRGVDVNTRDTDGFSPLLLAVRGRHPGVIGLLREAGASLSTQELEEAGTELCRLAYRADLEGLQVWWQAGADLGQPGYDGHSALHVAEAAGNLAVVAFLQSLEGAVGAQAPCPEVLPGV

SEQ ID NO: 38 - protein, 567 aa, Artificial Sequence
  Synthetic polypeptide
MARAVGPERRLLAVYTGGTIGMRSELGVLVPGTGLAAILRTLPMFHDEEHARARGLSEDTLVLPPASRNQRILYTVLECQPLFDSSDMTIAEWVCLAQTIKRHYEQYHGFVVIHGTDTMAFAASMLSFMLENLQKTVILTGAQVPIHALWSDGRENLLGALLMAGQYVIPEVCLFFQNQLFRGNRATKVDARRFAAFCSPNLLPLATVGADITINRELVRKVDGKAGLVVHSSMEQDVGLLRLYPGIPAALVRAFLQPPLKGVVMETFGSGNGPTKPDLLQELRVATERGLVIVNCTHCLQGAVTTDYAAGMAMAGAGVISGFDMTSEAALAKLSYVLGQPGLSLDVRKELLTKDLRGEMTLPTADLHQSSPPGSTLGQGVARLFSLFGCQEEDSVQDAVMPSLALALAHAGELEALQALMELGSDLRLKDSNGQTLLHVAARNGRDGVVTMLLHRGMDVNARDRDGLSPLLLAVQGRHRECIRLLRKAGACLSPQDLKDAGTELCRLASRADMEGLQAWGQAGADLQQPGYDGRSALCVAEAAGNQEVLALLRNLALVGPEVPPAI

SEQ ID NO: 39 - protein, 571 aa, Artificial Sequence
  Synthetic polypeptide
MARASGSERHLLLIYTGGTLGMQSKGGVLVPGPGLVTLLRTLPMFHDKEFARARGLSEDTLVLPPASRNQRILYTVLECQPLLDSSDMTIDDWIRIAKIIERHYEQYQGFVVIHGTDTMAFAASMLSFMLENLHKPVILTGAQVPIRVLWNDARENLLGALLVAGQYIIPEVCLFMNSQLFRGNRVTKVDSQKFEAFCSPNLSPLATVGADVTIAWDLVRKVKWKDPLVVHSSMEQDVGLLRLYPGIPASLVRAFLQPPLKGVVLETFGSGNGPSKPDLLQELRAAAERGLIMVNCSQCLRGSVTPGYATSLAGANIVSGLDMTSEAALAKLSYVLGLPELSLERRQELLAKDLRGEMTPPSVEERRPSLQGNTLGGGVSWLLSLSGSQEADALRNALVPSLACAAAHAGDVEALQALVELGSDLGLVDFNGQTPLHAAARGGHTEAVTMLLQRGVDVNTRDTDGFSPLLLAVRGRHPGVIGLLREAGASLSTQELEEAGTELCRLAYRADLEGLQVWWQAGADLGQPGYDGHSALHVAEAAGNLAVVAFLQSLEGAVGAQAPCPEVLPGV

SEQ ID NO: 40 - protein, 513 aa, Artificial Sequence
  Synthetic polypeptide
MARASGSERHLLLIYTGGTLGMQSKGGVLVPGPGLVTLLRTLPMFHDEEHARARGLSEDTLVLPPASRNQRILYTVLECQPLLDSSDMTIDDWIRIAKIIERHYEQYQGFVVIHGTDTMAFAASMLSFMLENLHKPVILTGAQVPIHALWSDGRENLLGALLVAGQYIIPEVCLFMNSQLFRGNRVTKVDSQKFEAFCSPNLSPLATVGADVTIAWDLVRKVKWKDPLVVHSSMEQDVGLLRLYPGIPASLVRAFLQPPLKGVVMETFGSGNGPTKPDLLQELRAAAERGLIMVNCSQCLRGSVTPGYATSLAGANIVSGLDMTSEAALAKLSYVLGLPELSLERRQELLAKDLRGEMTPPSVEERRPSLQGNTLGGGVSWLLSLSGSQEADALRNALVPSLACAAAHAGDVEALQALVELGSDLGLVDFNGQTPLHAAARGGHTEAVTMLLQRGVDVNTRDTDGFSPLLLAVRGRHPGVIGLLREAGASLSTQELEEAGTELCRLAYRADLE

SEQ ID NO: 41 - protein, 571 aa, Artificial Sequence
  Synthetic polypeptide
MARASGSERHLLLIYTGGTLGMQSKGGVLVPGPGLVTLLRTLPMFHDEEHARARGLSEDTLVLPPASRNQRILYTVLECQPLFDSSDMTIAEWVCLAQTIKRHYEQYHGFVVIHGTDTMAFAASMLSFMLENLHKPVILTGAQVPIHALWSDGRENLLGALLMAGQYVIPEVCLFFQNQLFRGNRATKVDARRFAAFCSPNLLPLATVGADVTIAWDLVRKVKWKDPLVVHSNMEHDVALLRLYPGIPAALVRAFLQPPLKGVVLETFGSGNGPSKPDLLQELRAAAERGLIMVNCSQCLRGSVTPGYATSLAGANIVSGLDMTSEAALAKLSYVLGLPELSLERRQELLAKDLRGEMTPPSVEERRPSLQGNTLGGGVSWLLSLSGSQEADALRNALVPSLACAAAHAGDVEALQALVELGSDLGLVDFNGQTPLHAAARGGHTEAVTMLLQRGVDVNTRDTDGFSPLLLAVRGRHPGVIGLLREAGASLSTQELEEAGTELCRLAYRADLEGLQVWWQAGADLGQPGYDGHSALHVAEAAGNLAVVAFLQSLEGAVGAQAPCPEVLPGV

SEQ ID NO: 42 - protein, 571 aa, Artificial Sequence
  Synthetic polypeptide
MARASGSERHLLLIYTGGTLGMQSKGGVLVPGPGLVTLLRTLPMFHDEEHARARGLSEDTLVLPPASRNQRILYTVLECQPLLDSSDMTIDDWIRIAKIIERHYEQYHGFVVIHGTDTMAFAASMLSFMLENLQKTVILTGAQVPIRVLWNDARENLLGALLVAGQYIIPEVCLFMSNQLFRGNRATKVDARRFAAFCSPNLSPLATVGADITINRELVRKVDGKAGLVVHSSMEQDVGLLRLYPGIPAALVRAFLQPPLKGVVMETFGSGNGPTKPDLLQELRVATERGLVIVNCTHCLQGAVTTGYATSLAGANIVSGLDMTSEAALAKLSYVLGLPELSLERRQELLAKDLRGEMTPPSVEERRPSLQGNTLGGGVSWLLSLSGSQEADALRNALVPSLACAAAHAGDVEALQALVELGSDLGLVDFNGQTPLHAAARGGHTEAVTMLLQRGVDVNTRDTDGFSPLLLAVRGRHPGVIGLLREAGASLSTQELEEAGTELCRLAYRADLEGLQVWWQAGADLGQPGYDGHSALHVAEAAGNLAVVAFLQSLEGAVGAQAPCPEVLPGV

SEQ ID NO: 43 - protein, 6 aa, Artificial Sequence
  Synthetic peptide
SEDTLV

SEQ ID NO: 44 - protein, 6 aa, Artificial Sequence
  Synthetic peptide
PDHALA

SEQ ID NO: 45 - protein, 369 aa, Artificial Sequence
  Synthetic polypeptide
MARASGSERHLLLIYTGGTLGMRSEGGVLVPGPGLVTLLRTLPMFHDEEFARARGLPDHALALPPASHGPRVLYTVLECQPLLDSSDMTIDDWIRIAQIIKRHYEQYQGFVVIHGTDTMAFAASMLSFMLENLQKPVILTGAQVPIRVLWNDARENLLGALLVAGQYIIPEVCLFMNSQLFRGNRVTKVDSQKFEAFCSPNLSPLATVGADVTIAWDLVRKVKWKDPLVVHSSMEHDVALLRLYPGIPASLVRAFLQPPLKGVVLETFGSGNGPSKPDLLQELRAAAERGLIMVNCSQCLRGSVTPGYATSLAGANIVSGLDMTSEAALAKLSYVLGLPELSLDRRQELLAKDLRGEMTPPSVEERRPS

SEQ ID NO: 46 - protein, 369 aa, Artificial Sequence
  Synthetic polypeptide
MARASGSERRLLLIYTGGTLGMRSEGGVLVPGPGLVTLLRTLPMFHDEEFARARGLPDHALALPPASHGPRVLYTVLECQPLLDSSDMTIAEWIRIAQIIKRHYEQYHGFVVIHGTDTMAFAASMLSFMLENLQKPVILTGAQVPIRVLWNDARENLLGALLVAGQYIIPEVCLFMNSQLFRGNRVTKVDSQKFEAFCSPNLSPLATVGADVTIAWDLVRKVKWKDPLVVHSSMEQDVALLRLYPGIPAALVRAFLQPPLKGVVLETFGSGNGPSKPDLLQELRAAAERGLIMVNCSQCLRGSVTPGYATSLAGANIVSGLDMTSEAALAKLSYVLGLPELSLDRRQELLAKDLRGEMTPPSVEERRPS

SEQ ID NO: 47 - protein, 369 aa, Artificial Sequence
  Synthetic polypeptide
MARASGSERRLLLIYTGGTLGMRSEGGVLVPGPGLVTLLRTLPMFHDEEFARARGLPDHALALPPASHGPRVLYTVLECQPLLDSSDMTIAEWIRIAQIIKRHYEQYHGFVVIHGTDTMAFAASMLSFMLENLQKPVILTGAQVPIHVLWNDARENLLGALLVAGQYIIPEVCLFMNSQLFRGNRVTKVDSQRFEAFCSPNLSPLATVGADVTIAWELVRKVKWKDPLVVHSSMEQDVALLRLYPGIPAALVRAFLQPPLKGVVLETFGSGNGPSKPDLLQELRAAAERGLIMVNCSQCLQGSVTPGYATSLAGANIVSGLDMTSEAALAKLSYVLGLPELSLDRRQELLAKDLRGEMTPPSVEERRPS

SEQ ID NO: 48 - protein, 369 aa, Artificial Sequence
  Synthetic polypeptide
MARASGSERHLLLIYTGGTLGMRSEGGVLVPGPGLVTLLRTLPMFHDEEFARARGLSEDTLVLPPASHGPRVLYTVLECQPLLDSSDMTIDDWIRIAQIIKRHYEQYQGFVVIHGTDTMAFAASMLSFMLENLQKPVILTGAQVPIRVLWNDARENLLGALLVAGQYIIPEVCLFMNSQLFRGNRVTKVDSQKFEAFCSPNLSPLATVGADVTIAWDLVRKVKWKDPLVVHSSMEHDVALLRLYPGIPASLVRAFLQPPLKGVVLETFGSGNGPSKPDLLQELRAAAERGLIMVNCSQCLRGSVTPGYATSLAGANIVSGLDMTSEAALAKLSYVLGLPELSLDRRQELLAKDLRGEMTPPSVEERRPS

SEQ ID NO: 49 - protein, 369 aa, Artificial Sequence
  Synthetic polypeptide
MARASGSERRLLLIYTGGTLGMRSEGGVLVPGPGLVTLLRTLPMFHDEEFARARGLSEDTLVLPPASHGPRVLYTVLECQPLLDSSDMTIAEWIRIAQIIKRHYEQYHGFVVIHGTDTMAFAASMLSFMLENLQKPVILTGAQVPIRVLWNDARENLLGALLVAGQYIIPEVCLFMNSQLFRGNRVTKVDSQKFEAFCSPNLSPLATVGADVTIAWDLVRKVKWKDPLVVHSSMEQDVALLRLYPGIPAALVRAFLQPPLKGVVLETFGSGNGPSKPDLLQELRAAAERGLIMVNCSQCLRGSVTPGYATSLAGANIVSGLDMTSEAALAKLSYVLGLPELSLDRRQELLAKDLRGEMTPPSVEERRPS

SEQ ID NO: 50 - protein, 369 aa, Artificial Sequence
  Synthetic polypeptide
MARASGSERRLLLIYTGGTLGMRSEGGVLVPGPGLVTLLRTLPMFHDEEFARARGLSEDTLVLPPASHGPRVLYTVLECQPLLDSSDMTIAEWIRIAQIIKRHYEQYHGFVVIHGTDTMAFAASMLSFMLENLQKPVILTGAQVPIHVLWNDARENLLGALLVAGQYIIPEVCLFMNSQLFRGNRVTKVDSQRFEAFCSPNLSPLATVGADVTIAWELVRKVKWKDPLVVHSSMEQDVALLRLYPGIPAALVRAFLQPPLKGVVLETFGSGNGPSKPDLLQELRAAAERGLIMVNCSQCLQGSVTPGYATSLAGANIVSGLDMTSEAALAKLSYVLGLPELSLDRRQELLAKDLRGEMTPPSVEERRPS

SEQ ID NO: 51 - protein, 369 aa, Artificial Sequence
  Synthetic polypeptide
MARASGSERHLLLIYTGGTLGMQSKGGVLVPGPGLVTLLRTLPMFHDKEFAQAQGLPDHALALPPASHGPRVLYTVLECQPLLDSSDMTIDDWIRIAKIIERHYEQYQGFVVIHGTDTMASGASMLSFMLENLHKPVILTGAQVPIRVLWNDARENLLGALLVAGQYIIPEVCLFMNSQLFRGNRVTKVDSQKFEAFASPNLSPLATVGADVTIAWDLVRKVKWKDPLVVHSNMEHDVALLRLYPGIPASLVRAFLQPPLKGVVLETFGSGNGPSKPDLLQELRAAAQRGLIMVNCSQCLRGSVTPGYATSLAGANIVSGLDMTSEAALAKLSYVLGLPELSLERRQELLAKDLRGEMTLPTADLHQSS

SEQ ID NO: 52 - protein, 369 aa, Artificial Sequence
  Synthetic polypeptide
MARASGSERHLLLIYTGGTLGMQSKGGVLVPGPGLVTLLRTLPMFHDKEFAQAQGLPDHALALPPASHGPRVLYTVLECQPLLDSSDMTIDDWIRIAKIIERHYEQYQGFVVIHGTDTMASGASMLSFMLENLHKPVILTGAQVPIRVLWNDARENLLGALLVAGQYIIPEVCLFMNSQLFRGNRVTKVDSQKFEAFSSPNLSPLATVGADVTIAWDLVRKVKWKDPLVVHSNMEHDVALLRLYPGIPASLVRAFLQPPLKGVVLETFGSGNGPSKPDLLQELRAAAQRGLIMVNCSQCLRGSVTPGYATSLAGANIVSGLDMTSEAALAKLSYVLGLPELSLERRQELLAKDLRGEMTLPTADLHQSS

SEQ ID NO: 53 - protein, 369 aa, Artificial Sequence
  Synthetic polypeptide
MARASGSERHLLLIYTGGTLGMQSKGGVLVPGPGLVTLLRTLPMFHDKEFAQAQGLPDHALALPPASHGPRVLYTVLECQPLLDSSDMTIDDWIRIAKIIERHYEQYQGFVVIHGTDTMASGASMLSFMLENLHKPVILTGAQVPIRVLWNDARENLLGALLVAGQYIIPEVCLFMNSQLFRGNRVTKVDSQKFEAFVSPNLSPLATVGADVTIAWDLVRKVKWKDPLVVHSNMEHDVALLRLYPGIPASLVRAFLQPPLKGVVLETFGSGNGPSKPDLLQELRAAAQRGLIMVNCSQCLRGSVTPGYATSLAGANIVSGLDMTSEAALAKLSYVLGLPELSLERRQELLAKDLRGEMTLPTADLHQSS

SEQ ID NO: 54 - protein, 369 aa, Artificial Sequence
  Synthetic polypeptide
MARASGSERHLLLIYTGGTLGMQSKGGVLVPGPGLVTLLRTLPMFHDKEFAQAQGLPDHALALPPASHGPRVLYTVLECQPLLDSSDMTIDDWIRIAKIIERHYEQYQGFVVIHGTDTMASGASMLSFMLENLHKPVILTGAQVPIRVLWNDARENLLGALLVAGQYIIPEVCLFMNSQLFRGNRVTKVDSQKFEAFASPNLSPLATVGADVTIAWDLVRKVKWCDPLVVHSNMEHDVALLRLYPGIPASLVRAFLQPPLKGVVLETFGSGNGPSKPDLLQELRAAAQRGLIMVNCSQCLRGSVTPGYATSLAGANIVSGLDMTSEAALAKLSYVLGLPELSLERRQELLAKDLRGEMTLPTADLHQSS

SEQ ID NO: 55 - protein, 369 aa, Artificial Sequence
  Synthetic polypeptide
MARASGSERHLLLIYTGGTLGMQSKGGVLVPGPGLVTLLRTLPMFHDKEFAQAQGLPDHALALPPASHGPRVLYTVLECQPLLDSSDMTIDDWIRIAKIIERHYEQYQGFVVIHGTDTMASGASMLSFMLENLHKPVILTGAQVPIRVLWNDARENLLGALLVAGQYIIPEVCLFMNSQLFRGNRVTKVDSQKFEAFASPNLSPLATVGADVTIAWDLVRKVKWCDPLVVHSNMEHDVALLRLYPGIPASLVRAFLQPPLKGVVLETFGSGNGPSKPDLLQELRAAAQRGLIMVNCSQCLRGSVTPGYATSLAGANIVSGLDMTSEAALAKLSYVLGLPCLSLERRQELLAKDLRGEMTLPTADLHQSS

SEQ ID NO: 56 - protein, 369 aa, Artificial Sequence
  Synthetic polypeptide
MARASGSERHLLLIYTGGTLGMQSKGGVLVPGPGLVTLLRTLPMFHDKCFAQAQGLPDHALALPPASHGPRVLYTVLECQPLLDSSDMTIDDWIRIAKIIERHYEQYQGFVVIHGTDTMASGASMLSFMLENLHKPVILTGAQVPIRVLWNDARENLLGALLVAGQYIIPEVCLFMNSQLFRGNRVTKVDSQKFEAFASPNLSPLATVGADVTIAWDLVRKVKWCDPLVVHSNMEHDVALLRLYPGIPASLVRAFLQPPLKGVVLETFGSGNGPSKPDLLQELRAAAQRGLIMVNCSQCLRGSVTPGYATSLAGANIVSGLDMTSEAALAKLSYVLGLPCLSLERRQELLAKDLRGEMTLPTADLHQSS

SEQ ID NO: 57 - protein, 369 aa, Artificial Sequence
  Synthetic polypeptide
MARASGSERHLLLIYTGGTLGMQSKGGVLVPGPGLVTLLRTLPMFHDKCFAQAQGLPDHALALPPASHGPRVLYTVLECQPLLDSSDMTIDDWIRIAKIIERHYEQYQGFVVIHGTDTMASGASMLSFMLENLHKPVILTGAQVPIRVLWNDARENLLGALLVAGQYIIPEVCLFMNSQLFRGNRVTKVDSQKFEAFASPNLSPLATVGADVTIAWDLVRKVKWCDPLVVHSNMEHDVALLRLYPGIPASLVRAFLCPPLKGVVLETFGSGNGPSKPDLLQELRAAAQRGLIMVNCSQCLRGSVTPGYATSLAGANIVSGLDMTSEAALAKLSYVLGLPCLSLERRQELLAKDLRGEMTLPTADLHQSS

SEQ ID NO: 58 - protein, 369 aa, Artificial Sequence
  Synthetic polypeptide
MARASGSERRLLLIYTGGTLGMRSEGGVLVPGPGLVTLLRTLPMFHDEEFARARGLSEDTLVLPPASHGPRVLYTVLECQPLLDSSDMTIAEWIRIAQIIKRHYEQYHGFVVIHGTDTMAFAASMLSFMLENLQKPVILTGAQVPIHVLWNDARENLLGALLVAGQYIIPEVCLFMNSQLFRGNRVTKVDSQRFEAFASPNLSPLATVGADVTIAWELVRKVKWKDPLVVHSSMEQDVALLRLYPGIPAALVRAFLQPPLKGVVLETFGSGNGPSKPDLLQELRAAAERGLIMVNCSQCLQGSVTPGYATSLAGANIVSGLDMTSEAALAKLSYVLGLPELSLDRRQELLAKDLRGEMTPPSVEERRPS

SEQ ID NO: 59 - protein, 369 aa, Artificial Sequence
  Synthetic polypeptide
MARASGSERRLLLIYTGGTLGMRSEGGVLVPGPGLVTLLRTLPMFHDEEFACARGLSEDTLVLPPASHGPRVLYTVLECQPLLDSSDMTIAEWIRIAQIIKRHYEQYHGFVVIHGTDTMAFAASMLSFMLENLQKPVILTGAQVPIHVLWNDARENLLGALLVAGQYIIPEVCLFMNSQLFRGNRVTKVDSQRFEAFASPNLSPLATVGADVTIAWELVRKVKWKDPLVVHSSMEQDVALLRLYPGIPAALVRAFLQPPLKGVVLETFGSGNGPSKPDLLQELRAAAERGLIMVNCSQCLQGSVTPGYATSLAGANIVSGLDMTSEAALAKLSYVLGLPELSLDRRQELLAKDLRGEMTPPSVEERRPS

SEQ ID NO: 60 - protein, 369 aa, Artificial Sequence
  Synthetic polypeptide
MARASGSERRLLLIYTGGTLGMRSEGGVLVPGPGLVTLLRTLPMFHDEEFACARGLSEDTLVLPPASHGPRVLYTVLECQPLLDSSDMTIAEWIRIAQIIKRHYEQYHGFVVIHGTDTMAFAASMLSFMLENLQKPVILTGAQVPIHVLWNDARENLLGALLVAGQYIIPEVCLFMNSQLFRGNRVTKVDSQRFEAFASPNLSPLATVGADVTIAWELVRKVKWCDPLVVHSSMEQDVALLRLYPGIPAALVRAFLQPPLKGVVLETFGSGNGPSKPDLLQELRAAAERGLIMVNCSQCLQGSVTPGYATSLAGANIVSGLDMTSEAALAKLSYVLGLPELSLDRRQELLAKDLRGEMTPPSVEERRPS

SEQ ID NO: 61 - protein, 369 aa, Artificial Sequence
  Synthetic polypeptide
MARASGSERRLLLIYTGGTLGMRSEGGVLVPGPGLVTLLRTLPMFHDEEFACARGLSEDTLVLPPASHGPRVLYTVLECQPLLDSSDMTIAEWIRIAQIIKRHYEQYHGFVVIHGTDTMAFAASMLSFMLENLQKPVILTGAQVPIHVLWNDARENLLGALLVAGQYIIPEVCLFMNSQLFRGNRVTKVDSQRFEAFASPNLSPLATVGADVTIAWELVRKVKWCDPLVVHSSMEQDVALLRLYPGIPAALVRAFLQPPLKGVVLETFGSGNGPSKPDLLQELRAAAERGLIMVNCSQCLQGSVTPGYATSLAGANIVSGLDMTSEAALAKLSYVLGLPCLSLDRRQELLAKDLRGEMTPPSVEERRPS

SEQ ID NO: 62 - protein, 369 aa, Artificial Sequence
  Synthetic polypeptide
MARASGSERRLLLIYTGGTLGMRSEGGVLVPGPGLVTLLRTLPMFHDEEFACARGLSEDTLVLPPASHGPRVLYTVLECQPLLDSSDMTIAEWIRIAQIIKRHYEQYHGFVVIHGTDTMAFAASMLSFMLENLQKPVILTGAQVPIHVLWNDARENLLGALLVAGQYIIPEVCLFMNSQLFRGNRVTKVDSQRFEAFASPNLSPLATVGADVTIAWELVRKVKWCDPLVVHSSMEQDVALLRLYPGIPAALVRAFLQPPLKGVVLETFGSGNGPSKPDLLCELRAAAERGLIMVNCSQCLQGSVTPGYATSLAGANIVSGLDMTSEAALAKLSYVLGLPCLSLDRRQELLAKDLRGEMTPPSVEERRPS

SEQ ID NO: 63 - protein, 369 aa, Artificial Sequence
  Synthetic polypeptide
MARASGSERHLLLIYTGGTLGMQSKGGVLVPGPGLVTLLRTLPMFHDKEFAQAKGLPDHALALPPASHGPRVLYTVLECQPLLDSSDMTIKDWIRIAKIIERHYEQYQGFVVIHGTDTMASGASMLSFMLENLHKPVILTGAQVPIRVLWNDARENLLGALLVAGQYIIPEVCLFMNSQLFRGNRVTKVDSQKFEAFCSPNLSPLATVGADVTIAWDLVRKVDWKDPLVVHSNMEHDVALLRLYPGIPASLVRAFLQPPLKGVVLETFGSGNGPSKPDLLQELRAAAQRGLIMVNCSQCLRGSVTPGYATKLAGANIVSGLDMTSEAALAKLSYVLGLPELSLERRQELLAKDLRGEMTLPTADLHQSS

SEQ ID NO: 64 - protein, 369 aa, Artificial Sequence
  Synthetic polypeptide
MARASGSERRLLLIYTGGTLGMRSEGGVLVPGPGLVTLLRTLPMFHDEEFARAKGLPDHALALPPASHGPRVLYTVLECQPLLDSSDMTIKEWIRIAQIIKRHYEQYHGFVVIHGTDTMAFAASMLSFMLENLQKPVILTGAQVPIHVLWNDARENLLGALLVAGQYIIPEVCLFMNSQLFRGNRVTKVDSQRFEAFASPNLSPLATVGADVTIAWELVRKVDWKDPLVVHSSMEQDVALLRLYPGIPAALVRAFLQPPLKGVVLETFGSGNGPSKPDLLQELRAAAERGLIMVNCSQCLQGSVTPGYATKLAGANIVSGLDMTSEAALAKLSYVLGLPELSLDRRQELLAKDLRGEMTPPSVEERRPS

SEQ ID NO: 65 - protein, 369 aa, Artificial Sequence
  Synthetic polypeptide
MARASGSERRLLLIYTGGTLGMRSEGGVLVPGPGLVTLLRTLPMFHDEEFARAKGLSEDTLVLPPASHGPRVLYTVLECQPLLDSSDMTIKEWIRIAQIIKRHYEQYHGFVVIHGTDTMAFAASMLSFMLENLQKPVILTGAQVPIHVLWNDARENLLGALLVAGQYIIPEVCLFMNSQLFRGNRVTKVDSQRFEAFASPNLSPLATVGADVTIAWELVRKVDWKDPLVVHSSMEQDVALLRLYPGIPAALVRAFLQPPLKGVVLETFGSGNGPSKPDLLQELRAAAERGLIMVNCSQCLQGSVTPGYATKLAGANIVSGLDMTSEAALAKLSYVLGLPELSLDRRQELLAKDLRGEMTPPSVEERRPS

SEQ ID NO: 66 - protein, 98 aa, Artificial Sequence
  Synthetic polypeptide
MSDSEVNQEAKPEVKPEVKPETHINLKVSDGSSEIFFKIKKTTPLRRLMEAFAKRQGKEMDSLRFLYDGIRIQADQTPEDLDMEDNDIIEAHREQIGG

SEQ ID NO: 67 - protein, 97 aa, Artificial Sequence
  Synthetic polypeptide
MSDQEAKPSTEDLGDKKEGEYIKLKVIGQDSSEIHFKVKMTTHLKKLKESYCQRQGVPMNSLRFLFEGQRIADNHTPKELGMEEEDVIEVYQEQTGG

SEQ ID NO: 68 - protein, 95 aa, Artificial Sequence
  Synthetic polypeptide
MADEKPKEGVKTENNDHINLKVAGQDGSVVQFKIKRHTPLSKLMKAYCERQGLSMRQIRFRFDGQPINETDTPAQLEMEDEDTIDVFQQQTGGVY

SEQ ID NO: 69 - protein, 103 aa, Artificial Sequence
  Synthetic polypeptide
MSEEKPKEGVKTENDHINLKVAGQDGSVVQFKIKRHTPLSKLMKAYCERQGLSMRQIRFRFDGQPINETDTPAQLEMEDEDTIDVFQQQTGGVPESSLAGHSF

SEQ ID NO: 70 - protein, 95 aa, Artificial Sequence
  Synthetic polypeptide
MANEKPTEEVKTENNNHINLKVAGQDGSVVQFKIKRQTPLSKLMKAYCEPRGLSMKQIRFRFGGQPISGTDKPAQLEMEDEDTIDVFQQPTGGVY

SEQ ID NO: 71 - protein, 20 aa, Artificial Sequence
  Synthetic peptide
QRLIEDICLPRWGCLWEDDF

SEQ ID NO: 72 - protein, 18 aa, Artificial Sequence
  Synthetic peptide
RLIEDICLPRWGCLWEDD

SEQ ID NO: 73 - protein, 15 aa, Artificial Sequence
  Synthetic peptide
RLIEDICLPRWGCLW

SEQ ID NO: 74 - protein, 468 aa, Artificial Sequence
  Synthetic polypeptide
MSDSEVNQEAKPEVKPEVKPETHINLKVSDGSSEIFFKIKKTTPLRRLMEAFAKRQGKEMDSLRFLYDGIRIQADQTPEDLDMEDNDIIEAHREQIGGHMARASGSERHLLLIYTGGTLGMQSKGGVLVPGPGLVTLLRTLPMFHDKEFAQAQGLPDHALALPPASHGPRVLYTVLEKQPLLDSSDMTIDDWIRIAKIIERHYEQYQGFVVIHGTDTMASGASMLSFMLENLHKPVILTGAQVPIRVLWNDARENLLGALLVAGQYIIPEVCLFMNSQLFRGNRVTKVDSQKFEAFASPNLSPLATVGADVTIAWDLVRKVKWKDPLVVHSNMEHDVALLRLYPGIPASLVRAFLQPPLKGVVLETFGSGNGPSKPDLLQELRAAAQRGLIMVNCSQCLRGSVTPGYATSLAGANIVSGLDMTSEAALAKLSYVLGLPELSLERRQELLAKDLRGEMTLPTADLHQSS

SEQ ID NO: 75 - protein, 467 aa, Artificial Sequence
  Synthetic polypeptide
MSDQEAKPSTEDLGDKKEGEYIKLKVIGQDSSEIHFKVKMTTHLKKLKESYCQRQGVPMNSLRFLFEGQRIADNHTPKELGMEEEDVIEVYQEQTGGHMARASGSERHLLLIYTGGTLGMQSKGGVLVPGPGLVTLLRTLPMFHDKEFAQAQGLPDHALALPPASHGPRVLYTVLEKQPLLDSSDMTIDDWIRIAKIIERHYEQYQGFVVIHGTDTMASGASMLSFMLENLHKPVILTGAQVPIRVLWNDARENLLGALLVAGQYIIPEVCLFMNSQLFRGNRVTKVDSQKFEAFASPNLSPLATVGADVTIAWDLVRKVKWKDPLVVHSNMEHDVALLRLYPGIPASLVRAFLQPPLKGVVLETFGSGNGPSKPDLLQELRAAAQRGLIMVNCSQCLRGSVTPGYATSLAGANIVSGLDMTSEAALAKLSYVLGLPELSLERRQELLAKDLRGEMTLPTADLHQSS

SEQ ID NO: 76 - protein, 386 aa, Artificial Sequence
  Synthetic polypeptide
RLIEDICLPRWGCLWEDDARASGSERHLLLIYTGGTLGMQSKGGVLVPGPGLVTLLRTLPMFHDKEFAQAQGLPDHALALPPASHGPRVLYTVLECQPLLDSSDMTIDDWIRIAKIIERHYEQYQGFVVIHGTDTMASGASMLSFMLENLHKPVILTGAQVPIRVLWNDARENLLGALLVAGQYIIPEVCLFMNSQLFRGNRVTKVDSQKFEAFASPNLSPLATVGADVTIAWDLVRKVKWKDPLVVHSNMEHDVALLRLYPGIPASLVRAFLQPPLKGVVLETFGSGNGPSKPDLLQELRAAAQRGLIMVNCSQCLRGSVTPGYATSLAGANIVSGLDMTSEAALAKLSYVLGLPELSLERRQELLAKDLRGEMTLPTADLHQSS

SEQ ID NO: 77 - protein, 387 aa, Artificial Sequence
  Synthetic polypeptide
MARASGSERHLLLIYTGGTLGMQSKGGVLVPGPGLVTLLRTLPMFHDKEFAQAQGLPDHALALPPASHGPRVLYTVLECQPLLDSSDMTIDDWIRIAKIIERHYEQYQGFVVIHGTDTMASGASMLSFMLENLHKPVILTGAQVPIRVLWNDARENLLGALLVAGQYIIPEVCLFMNSQLFRGNRVTKVDSQKFEAFASPNLSPLATVGADVTIAWDLVRKVKWKDPLVVHSNMEHDVALLRLYPGIPASLVRAFLQPPLKGVVLETFGSGNGPSKPDLLQELRAAAQRGLIMVNCSQCLRGSVTPGYATSLAGANIVSGLDMTSEAALAKLSYVLGLPELSLERRQELLAKDLRGEMTLPTADLHQSSRLIEDICLPRWGCLWEDD

SEQ ID NO: 78 - protein, 486 aa, Artificial Sequence
  Synthetic polypeptide
MSDSEVNQEAKPEVKPEVKPETHINLKVSDGSSEIFFKIKKTTPLRRLMEAFAKRQGKEMDSLRFLYDGIRIQADQTPEDLDMEDNDIIEAHREQIGGHMARASGSERHLLLIYTGGTLGMQSKGGVLVPGPGLVTLLRTLPMFHDKEFAQAQGLPDHALALPPASHGPRVLYTVLECQPLLDSSDMTIDDWIRIAKIIERHYEQYQGFVVIHGTDTMASGASMLSFMLENLHKPVILTGAQVPIRVLWNDARENLLGALLVAGQYIIPEVCLFMNSQLFRGNRVTKVDSQKFEAFASPNLSPLATVGADVTIAWDLVRKVKWKDPLVVHSNMEHDVALLRLYPGIPASLVRAFLQPPLKGVVLETFGSGNGPSKPDLLQELRAAAQRGLIMVNCSQCLRGSVTPGYATSLAGANIVSGLDMTSEAALAKLSYVLGLPELSLERRQELLAKDLRGEMTLPTADLHQSSRLIEDICLPRWGCLWEDD

SEQ ID NO: 79 - protein, 485 aa, Artificial Sequence
  Synthetic polypeptide
MSDQEAKPSTEDLGDKKEGEYIKLKVIGQDSSEIHFKVKMTTHLKKLKESYCQRQGVPMNSLRFLFEGQRIADNHTPKELGMEEEDVIEVYQEQTGGHMARASGSERHLLLIYTGGTLGMQSKGGVLVPGPGLVTLLRTLPMFHDKEFAQAQGLPDHALALPPASHGPRVLYTVLECQPLLDSSDMTIDDWIRIAKIIERHYEQYQGFVVIHGTDTMASGASMLSFMLENLHKPVILTGAQVPIRVLWNDARENLLGALLVAGQYIIPEVCLFMNSQLFRGNRVTKVDSQKFEAFASPNLSPLATVGADVTIAWDLVRKVKWKDPLVVHSNMEHDVALLRLYPGIPASLVRAFLQPPLKGVVLETFGSGNGPSKPDLLQELRAAAQRGLIMVNCSQCLRGSVTPGYATSLAGANIVSGLDMTSEAALAKLSYVLGLPELSLERRQELLAKDLRGEMTLPTADLHQSSRLIEDICLPRWGCLWEDD

SEQ ID NO: 80 - protein, 167 aa, Artificial Sequence
  Synthetic polypeptide
RERGPQRVAAHITGTRGRSNTLSSPNSKNEKALGRKINSWESSRSGHSFLSNLHLRNGELVIHEKGFYYIYSQTYFRFQEEIKENTKNDKQMVQYIYKYTSYPDPILLMKSARNSCWSKDAEYGLYSIYQGGIFELKENDRIFVSVTNEHLIDMDHEASFFGAFLVG

SEQ ID NO: 81 - protein, 16 aa, Artificial Sequence
  Synthetic peptide
  MISC_FEATURE (5)..(16): Residue may be present or absent
GGGSGGGSGGGSGGGS

SEQ ID NO: 82 - protein, 24 aa, Artificial Sequence
  Synthetic peptide
  MISC_FEATURE (10)..(24): Residue may be present or absent
GGGSGGGGSGGGGSGGGGSGGGGS

SEQ ID NO: 83 - protein, 24 aa, Artificial Sequence
  Synthetic peptide
GGGSGGGGSGGGGSGGGGSGGGGS

SEQ ID NO: 84 - protein, 19 aa, Artificial Sequence
  Synthetic peptide
SGSGSGSGSGSGSGSGSGS

SEQ ID NO: 85 - protein, 27 aa, Artificial Sequence
  Synthetic peptide
GYIPEAPRDGQAYVRKDGEWVLLSTFL

SEQ ID NO: 86 - protein, 369 aa, Artificial Sequence
  Synthetic polypeptide
MARASGKERRLLLIYTGGTLGMRSEGGVLVPGPGLVTLLRTLPMFHDEEFARKKGLKKDTLVLPPASHGPRVLYTVLECQPLLDSSDMTIAEWIRIAKIIKRHYEKYHGFVVIHGTDTMAFAASMLSFMLENLQKPVILTGAQVPIHVLWNDARENLLGALLVAGQYIIPEVCLFMNSQLFRGNRVTKVDSQRFEAFASPNLSPLATVGADVTIAWELVRKVKWKDPLVVHSKMEQDVALLRLYPGIPAKLVRAFLKPPLKGVVLETFGSGNGPSKPDLLKELRAAAERGLIMVNCSQCLQGSVTPGYATKLAGANIVSGLDMTSEAALAKLSYVLGLPKLSLDRRQELLAKDLRGEMTPPSVEERRPS

SEQ ID NO: 87 - protein, 503 aa, Artificial Sequence
  Synthetic polypeptide
RERGPQRVAAHITGTRGRSNTLSSPNSKNEKALGRKINSWESSRSGHSFLSNLHLRNGELVIHEKGFYYIYSQTYFRFQEEIKENTKNDKQMVQYIYKYTSYPDPILLMKSARNSCWSKDAEYGLYSIYQGGIFELKENDRIFVSVTNEHLIDMDHEASFFGAFLVGGRERGPQRVAAHITGTRGRSNTLSSPNSKNEKALGRKINSWESSRSGHSFLSNLHLRNGELVIHEKGFYYIYSQTYFRFQEEIKENTKNDKQMVQYIYKYTSYPDPILLMKSARNSCWSKDAEYGLYSIYQGGIFELKENDRIFVSVTNEHLIDMDHEASFFGAFLVGSRERGPQRVAAHITGTRGRSNTLSSPNSKNEKALGRKINSWESSRSGHSFLSNLHLRNGELVIHEKGFYYIYSQTYFRFQEEIKENTKNDKQMVQYIYKYTSYPDPILLMKSARNSCWSKDAEYGLYSIYQGGIFELKENDRIFVSVTNEHLIDMDHEASFFGAFLVG

SEQ ID NO: 88 - protein, 503 aa, Artificial Sequence
  Synthetic polypeptide
RERGPQRVAAHITGTRGRSNTLSSPNSKNEKALGRKINSWESSRSGHSFLSNLHLRNGELVIHEKGFYYIYSQTYFRFQEEIKENTKNDKQMVQYIYKYTSYPDPILLMKSARNSCWSKDAEYGLYSIYQGGIFELKENDRIFVSVTNEHLIDMDHEASFFGAFLVGSRERGPQRVAAHITGTRGRSNTLSSPNSKNEKALGRKINSWESSRSGHSFLSNLHLRNGELVIHEKGFYYIYSQTYFRFQEEIKENTKNDKQMVQYIYKYTSYPDPILLMKSARNSCWSKDAEYGLYSIYQGGIFELKENDRIFVSVTNEHLIDMDHEASFFGAFLVGSRERGPQRVAAHITGTRGRSNTLSSPNSKNEKALGRKINSWESSRSGHSFLSNLHLRNGELVIHEKGFYYIYSQTYFRFQEEIKENTKNDKQMVQYIYKYTSYPDPILLMKSARNSCWSKDAEYGLYSIYQGGIFELKENDRIFVSVTNEHLIDMDHEASFFGAFLVG

SEQ ID NO: 89 - protein, 874 aa, Artificial Sequence
  Synthetic polypeptide
MARASGSERRLLLIYTGGTLGMRSEGGVLVPGPGLVTLLRTLPMFHDEEFARARGLSEDTLVLPPASHGPRVLYTVLECQPLLDSSDMTIAEWIRIAQIIKRHYEQYHGFVVIHGTDTMAFAASMLSFMLENLQKPVILTGAQVPIHVLWNDARENLLGALLVAGQYIIPEVCLFMNSQLFRGNRVTKVDSQRFEAFASPNLSPLATVGADVTIAWELVRKVKWKDPLVVHSSMEQDVALLRLYPGIPAALVRAFLQPPLKGVVLETFGSGNGPSKPDLLQELRAAAERGLIMVNCSQCLQGSVTPGYATSLAGANIVSGLDMTSEAALAKLSYVLGLPELSLDRRQELLAKDLRGEMTPPSVEERRPSTSRERGPQRVAAHITGTRGRSNTLSSPNSKNEKALGRKINSWESSRSGHSFLSNLHLRNGELVIHEKGFYYIYSQTYFRFQEEIKENTKNDKQMVQYIYKYTSYPDPILLMKSARNSCWSKDAEYGLYSIYQGGIFELKENDRIFVSVTNEHLIDMDHEASFFGAFLVGGRERGPQRVAAHITGTRGRSNTLSSPNSKNEKALGRKINSWESSRSGHSFLSNLHLRNGELVIHEKGFYYIYSQTYFRFQEEIKENTKNDKQMVQYIYKYTSYPDPILLMKSARNSCWSKDAEYGLYSIYQGGIFELKENDRIFVSVTNEHLIDMDHEASFFGAFLVGSRERGPQRVAAHITGTRGRSNTLSSPNSKNEKALGRKINSWESSRSGHSFLSNLHLRNGELVIHEKGFYYIYSQTYFRFQEEIKENTKNDKQMVQYIYKYTSYPDPILLMKSARNSCWSKDAEYGLYSIYQGGIFELKENDRIFVSVTNEHLIDMDHEASFFGAFLVG

SEQ ID NO: 90 - protein, 883 aa, Artificial Sequence
  Synthetic polypeptide
SERRLLLIYTGGTLGMRSEGGVLVPGPGLVTLLRTLPMFHDEEFARARGLSEDTLVLPPASHGPRVLYTVLECQPLLDSSDMTIAEWIRIAQIIKRHYEQYHGFVVIHGTDTMAFAASMLSFMLENLQKPVILTGAQVPIHVLWNDARENLLGALLVAGQYIIPEVCLFMNSQLFRGNRVTKVDSQRFEAFASPNLSPLATVGADVTIAWELVRKVKWKDPLVVHSSMEQDVALLRLYPGIPAALVRAFLQPPLKGVVLETFGSGNGPSKPDLLQELRAAAERGLIMVNCSQCLQGSVTPGYATSLAGANIVSGLDMTSEAALAKLSYVLGLPELSLDRRQELLAKDLRGEMTPPSVEERRPSLQGNTLGGGVSWLLSTSRERGPQRVAAHITGTRGRSNTLSSPNSKNEKALGRKINSWESSRSGHSFLSNLHLRNGELVIHEKGFYYIYSQTYFRFQEEIKENTKNDKQMVQYIYKYTSYPDPILLMKSARNSCWSKDAEYGLYSIYQGGIFELKENDRIFVSVTNEHLIDMDHEASFFGAFLVGSRERGPQRVAAHITGTRGRSNTLSSPNSKNEKALGRKINSWESSRSGHSFLSNLHLRNGELVIHEKGFYYIYSQTYFRFQEEIKENTKNDKQMVQYIYKYTSYPDPILLMKSARNSCWSKDAEYGLYSIYQGGIFELKENDRIFVSVTNEHLIDMDHEASFFGAFLVGSRERGPQRVAAHITGTRGRSNTLSSPNSKNEKALGRKINSWESSRSGHSFLSNLHLRNGELVIHEKGFYYIYSQTYFRFQEEIKENTKNDKQMVQYIYKYTSYPDPILLMKSARNSCWSKDAEYGLYSIYQGGIFELKENDRIFVSVTNEHLIDMDHEASFFGAFLVG

SEQ ID NO: 91 - protein, 872 aa, Artificial Sequence
  Synthetic polypeptide
RERGPQRVAAHITGTRGRSNTLSSPNSKNEKALGRKINSWESSRSGHSFLSNLHLRNGELVIHEKGFYYIYSQTYFRFQEEIKENTKNDKQMVQYIYKYTSYPDPILLMKSARNSCWSKDAEYGLYSIYQGGIFELKENDRIFVSVTNEHLIDMDHEASFFGAFLVGSRERGPQRVAAHITGTRGRSNTLSSPNSKNEKALGRKINSWESSRSGHSFLSNLHLRNGELVIHEKGFYYIYSQTYFRFQEEIKENTKNDKQMVQYIYKYTSYPDPILLMKSARNSCWSKDAEYGLYSIYQGGIFELKENDRIFVSVTNEHLIDMDHEASFFGAFLVGSRERGPQRVAAHITGTRGRSNTLSSPNSKNEKALGRKINSWESSRSGHSFLSNLHLRNGELVIHEKGFYYIYSQTYFRFQEEIKENTKNDKQMVQYIYKYTSYPDPILLMKSARNSCWSKDAEYGLYSIYQGGIFELKENDRIFVSVTNEHLIDMDHEASFFGAFLVGMARASGSERRLLLIYTGGTLGMRSEGGVLVPGPGLVTLLRTLPMFHDEEFARARGLSEDTLVLPPASHGPRVLYTVLECQPLLDSSDMTIAEWIRIAQIIKRHYEQYHGFVVIHGTDTMAFAASMLSFMLENLQKPVILTGAQVPIHVLWNDARENLLGALLVAGQYIIPEVCLFMNSQLFRGNRVTKVDSQRFEAFASPNLSPLATVGADVTIAWELVRKVKWKDPLVVHSSMEQDVALLRLYPGIPAALVRAFLQPPLKGVVLETFGSGNGPSKPDLLQELRAAAERGLIMVNCSQCLQGSVTPGYATSLAGANIVSGLDMTSEAALAKLSYVLGLPELSLDRRQELLAKDLRGEMTPPSVEERRPS

SEQ ID NO: 92 - protein, 891 aa, Artificial Sequence
  Synthetic polypeptide
RERGPQRVAAHITGTRGRSNTLSSPNSKNEKALGRKINSWESSRSGHSFLSNLHLRNGELVIHEKGFYYIYSQTYFRFQEEIKENTKNDKQMVQYIYKYTSYPDPILLMKSARNSCWSKDAEYGLYSIYQGGIFELKENDRIFVSVTNEHLIDMDHEASFFGAFLVGSRERGPQRVAAHITGTRGRSNTLSSPNSKNEKALGRKINSWESSRSGHSFLSNLHLRNGELVIHEKGFYYIYSQTYFRFQEEIKENTKNDKQMVQYIYKYTSYPDPILLMKSARNSCWSKDAEYGLYSIYQGGIFELKENDRIFVSVTNEHLIDMDHEASFFGAFLVGSRERGPQRVAAHITGTRGRSNTLSSPNSKNEKALGRKINSWESSRSGHSFLSNLHLRNGELVIHEKGFYYIYSQTYFRFQEEIKENTKNDKQMVQYIYKYTSYPDPILLMKSARNSCWSKDAEYGLYSIYQGGIFELKENDRIFVSVTNEHLIDMDHEASFFGAFLVGSGSGSGSGSGSGSGSGSGSMARASGSERRLLLIYTGGTLGMRSEGGVLVPGPGLVTLLRTLPMFHDEEFARARGLSEDTLVLPPASHGPRVLYTVLECQPLLDSSDMTIAEWIRIAQIIKRHYEQYHGFVVIHGTDTMAFAASMLSFMLENLQKPVILTGAQVPIHVLWNDARENLLGALLVAGQYIIPEVCLFMNSQLFRGNRVTKVDSQRFEAFASPNLSPLATVGADVTIAWELVRKVKWKDPLVVHSSMEQDVALLRLYPGIPAALVRAFLQPPLKGVVLETFGSGNGPSKPDLLQELRAAAERGLIMVNCSQCLQGSVTPGYATSLAGANIVSGLDMTSEAALAKLSYVLGLPELSLDRRQELLAKDLRGEMTPPSVEERRPS

SEQ ID NO: 93 - protein, 387 aa, Artificial Sequence
  Synthetic polypeptide
MARASGSERRLLLIYTGGTLGMRSEGGVLVPGPGLVTLLRTLPMFHDEEFARARGLSEDTLVLPPASHGPRVLYTVLECQPLLDSSDMTIAEWIRIAQIIKRHYEQYHGFVVIHGTDTMAFAASMLSFMLENLQKPVILTGAQVPIHVLWNDARENLLGALLVAGQYIIPEVCLFMNSQLFRGNRVTKVDSQRFEAFASPNLSPLATVGADVTIAWELVRKVKWKRLIEDICLPRWGCLWEDDDPLVVHSSMEQDVALLRLYPGIPAALVRAFLQPPLKGVVLETFGSGNGPSKPDLLQELRAAAERGLIMVNCSQCLQGSVTPGYATSLAGANIVSGLDMTSEAALAKLSYVLGLPELSLDRRQELLAKDLRGEMTPPSVEERRPS

SEQ ID NO: 94 - protein, 387 aa, Artificial Sequence
  Synthetic polypeptide
MARASGSERRLLLIYTGGTLGMRSEGGVLVPGPGLVTLLRTLPMFHDEEFARARGLSEDTLVLPPASHGPRVLYTVLECQPLLDSSDMTIAEWIRIAQIIKRHYEQYHGFVVIHGTDTMAFAASMLSFMLENLQKPVILTGAQVPIHVLWNDARENLLGALLVAGQYIIPEVCLFMNSQLFRGNRVTKVDSQRFEAFASPNLSPLATVGADVTIAWELVRKVKWKDPLVVHSSMEQDVALLRLYPGIPAALVRAFLQPPLKGVVLETFGSGNGPSKPDLLQELRAAAERGLIMVNCSQCLQGSVTPGYATSLAGANIVSGLDMTSEAALAKLSYVLGLPERLIEDICLPRWGCLWEDDLSLDRRQELLAKDLRGEMTPPSVEERRPS